European Patent Specification EP 3 774 898 B1, published August 26, 2026. Title: ANTI-CD27 ANTIBODIES AND USE THEREOF. Applicant: DINGFU BIOTARGET CO.,LTD. The sequence listing filed with the application follows.

SEQUENCE LISTING (152 sequences)

SEQ ID NO: 1 - protein, 122 aa, Artificial Sequence
  1A8 VH
EVQLQESGAELVKPGASVKLSCKASGYSFTSSWMHWVKQRPGQGLEWIGMIHPDSGFTNYNEKFKSKATLTVDKSSSTAYMRLSSLTSEDSAVYYCARTSYYDTSYTSMDFWGQGNSVTVSS

SEQ ID NO: 2 - DNA, 366 bp, Artificial Sequence
  1A8 VH nucleotide
gaggtgcagctgcaggagtctggggctgaattggtaaagcctggggcttcagtgaagttgtcctgcaaggcttctggctacagtttcaccagctcctggatgcactgggtgaagcagaggcctggacaaggccttgagtggattggaatgattcatcctgatagtggttttactaactacaatgagaagttcaagagcaaggccacactgactgtagacaaatcctccagcacagcctacatgcgcctcagcagcctgacatctgaggactctgcggtctattactgtgcaaggacctcttactacgatactagctacacttctatggacttctggggtcaaggaaactcagtcaccgtctcctca

SEQ ID NO: 3 - protein, 107 aa, Artificial Sequence
  1A8VL
DIVLTQSPAILSVSPGERVSFSCRASQSIGTSIHWYQQRTNGSPRLLIKYASESISGIPSRFSGSGSGTDFTLSINSVESEDIADYYCQQSNSWPLTFGAGTKLELK

SEQ ID NO: 4 - DNA, 321 bp, Artificial Sequence
  1A8VL nucleotide
gatattgtgctgacccagtctccagccatcctgtctgtgagtccaggagaaagagtcagtttctcctgcagggccagtcagagcattggcacaagcatacattggtatcagcaaagaacaaatggttctccaaggcttctcataaagtatgcttctgagtctatctctgggatcccttccaggtttagtggcagtggatcagggacagattttactcttagcatcaacagtgtggagtctgaagatattgcagattattactgtcaacaaagtaatagctggccactcacgttcggtgctgggaccaagctggagctgaaa

SEQ ID NO: 5 - protein, 5 aa, Artificial Sequence
  1A8 HCDR1
SSWMH

SEQ ID NO: 6 - protein, 17 aa, Artificial Sequence
  1A8 HCDR2
MIHPDSGFTNYNEKFKS

SEQ ID NO: 7 - protein, 13 aa, Artificial Sequence
  1A8 HCDR3
TSYYDTSYTSMDF

SEQ ID NO: 8 - protein, 11 aa, Artificial Sequence
  1A8 LCDR1
RASQSIGTSIH

SEQ ID NO: 9 - protein, 7 aa, Artificial Sequence
  1A8 LCDR2
YASESIS

SEQ ID NO: 10 - protein, 9 aa, Artificial Sequence
  1A8 LCDR3
QQSNSWPLT

SEQ ID NO: 11 - protein, 120 aa, Artificial Sequence
  2B8 VH
EVQLQESGGGLVQPKGSLKLSCAASGFNFNTYTMNWVRQAPGKGLEWVARIRYKSNNYATYYADSVKDRFTISRDDSESILYLQMNNLRTDDTAIYFCVRELGLWYFDVWGAGTTVTVSS

SEQ ID NO: 12 - DNA, 360 bp, Artificial Sequence
  2B8 VH nucleotide
gaggtgcagctgcaggagtctggtggaggattggtgcagcctaaagggtcattgaaactctcatgtgcagcctctggattcaacttcaatacctacaccatgaactgggtccgccaggctccaggaaagggtttggaatgggttgctcgcataagatataaaagtaataattatgcaacatattatgccgattcagtgaaagacagattcaccatctccagagatgattcagaaagcatcctctatctgcaaatgaacaacttgagaactgacgacacagccatttatttctgtgtgagggaactgggactgtggtacttcgatgtctggggcgcagggaccacggtcaccgtctcctca

SEQ ID NO: 13 - protein, 107 aa, Artificial Sequence
  2B8VL
DIVMTQSPSYLAASPGETITINCRASKSISKYLAWYREKPGKTNNLLIYSGSTLQSGIPSRFSGSGSGTDFTLTISSLEPEDFAMYYCQQHNEYPLTFGAGTKLELK

SEQ ID NO: 14 - DNA, 321 bp, Artificial Sequence
  2B8VL nucleotide
gacattgtgatgacccagtctccatcttatcttgctgcatctcctggagaaaccattactataaattgcagggcaagtaagagcattagcaaatatttagcctggtatcgagagaaacctgggaaaactaataatcttcttatctactctggatccactttgcaatctggaattccatcaaggttcagtggcagtggatctggtacagatttcactctcaccatcagtagcctggagcctgaagattttgcaatgtattactgtcaacagcataatgaatacccgctcacgttcggtgctgggaccaagctggagctgaaa

SEQ ID NO: 15 - protein, 5 aa, Artificial Sequence
  2B8 HCDR1
TYTMN

SEQ ID NO: 16 - protein, 19 aa, Artificial Sequence
  2B8 HCDR2
RIRYKSNNYATYYADSVKD

SEQ ID NO: 17 - protein, 9 aa, Artificial Sequence
  2B8 HCDR3
ELGLWYFDV

SEQ ID NO: 18 - protein, 11 aa, Artificial Sequence
  2B8 LCDR1
RASKSISKYLA

SEQ ID NO: 19 - protein, 7 aa, Artificial Sequence
  2B8 LCDR2
SGSTLQS

SEQ ID NO: 20 - protein, 9 aa, Artificial Sequence
  2B8 LCDR3
QQHNEYPLT

SEQ ID NO: 21 - protein, 116 aa, Artificial Sequence
  2E7 VH
EVQLQESGPELKKPGETVKISCKASGYTFTTYGMSWVKQAPGKGLQWMGWINTNSGVPTYVEDFKGRFAFSLESSANTAYLQINNLKNEDTAIYFCTREGDALDYWGQGTSVTVSS

SEQ ID NO: 22 - DNA, 348 bp, Artificial Sequence
  2E7 VH nucleotide
gaggtgcagctgcaggagtctggacctgagctgaagaagcctggagagacagtcaagatctcctgcaaggcttctgggtataccttcacaacctatggaatgagctgggtgaaacaggctccaggaaagggtttacagtggatgggctggataaacaccaactctggagtgccaacctatgttgaggacttcaagggacggtttgccttctctttggaatcctctgccaacactgcctatttgcagatcaacaacctcaaaaatgaggacacggctatatacttctgtacaagagagggggatgctctggactactggggtcaaggaacctcagtcaccgtctcctca

SEQ ID NO: 23 - protein, 107 aa, Artificial Sequence
  2E7VL
DIVMTQSTAIMSASPGEKVTMTCSASSSVSYMHWYQQKSGTSPRRWIYDTSRLASGVPARFSGSGSGTSYSLTISSMEAEDAATYYCQQWSNTPPFTFGAGTKLELK

SEQ ID NO: 24 - DNA, 321 bp, Artificial Sequence
  2E7VL nucleotide
gatattgtgatgacacaatctacagcaatcatgtctgcatctccaggggagaaggtcaccatgacctgcagtgccagctcaagtgtaagttacatgcactggtaccagcagaagtcaggcacctcccccagaagatggatttatgacacatccagactggcttctggagtccctgctcgcttcagtggcagtgggtctgggacctcttactctctcacaatcagcagcatggaggctgaagatgctgccacttattactgccagcagtggagtaataccccacccttcacgttcggtgctgggaccaagttggagctgaaa

SEQ ID NO: 25 - protein, 5 aa, Artificial Sequence
  2E7 HCDR1
TYGMS

SEQ ID NO: 26 - protein, 17 aa, Artificial Sequence
  2E7 HCDR2
WINTNSGVPTYVEDFKG

SEQ ID NO: 27 - protein, 7 aa, Artificial Sequence
  2E7 HCDR3
EGDALDY

SEQ ID NO: 28 - protein, 10 aa, Artificial Sequence
  2E7 LCDR1
SASSSVSYMH

SEQ ID NO: 29 - protein, 7 aa, Artificial Sequence
  2E7 LCDR2
DTSRLAS

SEQ ID NO: 30 - protein, 10 aa, Artificial Sequence
  2E7 LCDR3
QQWSNTPPFT

SEQ ID NO: 31 - protein, 116 aa, Artificial Sequence
  3E7 VH
QIQLVQSGPELKKPGETVKISCKASGYTFTTYGMSWVKQAPGKGLHWMGWINTHSGAPTYVDDFKGRFAFSLETSASTAFLQINNLINEDTATYFCAREGDALDYWGQGTSVTVSS

SEQ ID NO: 32 - DNA, 348 bp, Artificial Sequence
  3E7 VH nucleotide
cagatccagctggtgcagagcggaccagaactgaagaagccaggagagacagtcaagatctcctgcaaggcttctggatatacgttcacaacctatggaatgagctgggtgaaacaggctccaggaaagggtttgcactggatgggctggataaacacccactctggagcgccaacatatgttgatgacttcaagggacggtttgccttctctttggaaacctctgccagcactgcctttttgcagatcaacaacctcataaatgaggacacggctacatatttctgtgcaagagagggggatgctctggactactggggtcaaggaacctcagtcaccgtctcctca

SEQ ID NO: 33 - protein, 107 aa, Artificial Sequence
  3E7VL
DIVMTQTTAIMSAFPGEKVTMTCSASSSVSYMHWYQQKSGTSPKRWIYDTSKLASGVPVRFSGSGSGTSYSLTISNMEAEDAATYYCQQWSRNPPFTFGAGTKLELK

SEQ ID NO: 34 - DNA, 321 bp, Artificial Sequence
  3E7VL nucleotide
gacattgtgatgacccaaactacagcaatcatgtctgcatttccaggggagaaggtcaccatgacctgcagtgccagctcaagtgtaagttacatgcactggtaccagcagaagtcaggcacctcccccaaaagatggatttatgacacatccaaactggcttctggagtccctgttcgcttcagtggcagtgggtctgggacctcttactctctcacaatcagcaacatggaggctgaagatgctgccacttattattgccagcagtggagtcgtaacccacccttcacgttcggtgctgggaccaagctggagctgaaa

SEQ ID NO: 35 - protein, 5 aa, Artificial Sequence
  3E7 HCDR1
TYGMS

SEQ ID NO: 36 - protein, 17 aa, Artificial Sequence
  3E7 HCDR2
WINTHSGAPTYVDDFKG

SEQ ID NO: 37 - protein, 7 aa, Artificial Sequence
  3E7 HCDR3
EGDALDY

SEQ ID NO: 38 - protein, 10 aa, Artificial Sequence
  3E7 LCDR1
SASSSVSYMH

SEQ ID NO: 39 - protein, 7 aa, Artificial Sequence
  3E7 LCDR2
DTSKLAS

SEQ ID NO: 40 - protein, 10 aa, Artificial Sequence
  3E7 LCDR3
QQWSRNPPFT

SEQ ID NO: 41 - protein, 121 aa, Artificial Sequence
  3B8 VH
QVQLQESGPGLVAPSQSLSITCTVSGFSLTNYAVSWVRQPPGKGLEWLGVIWGDGTTNYHSALISRLIISKDNSKSQVFLKLNSLQTDDTATYYCAKEGDYGDYVGWFAYWGQGTLVTVSA

SEQ ID NO: 42 - DNA, 363 bp, Artificial Sequence
  3B8 VH nucleotide
caggtccagctgcaggagtcaggacctggcctggtggcgccctcacagagcctgtccatcacatgcactgtctcagggttctcattaaccaactatgctgtaagctgggttcgccagcctccaggaaagggtctggagtggctgggagtaatatggggtgacgggaccacaaattatcattcagctctcatatccagactgattatcagcaaggataactccaagagccaagttttcttaaaactgaacagtctgcaaactgatgacacagccacgtactactgtgccaaagagggcgactatggtgactacgtaggctggtttgcttactggggccaagggactctggtcactgtctctgca

SEQ ID NO: 43 - protein, 111 aa, Artificial Sequence
  3B8VL
DIVLTQSPASLAVSLGQRATISCRASESVEYYGTSLMQWYQQKPGQPPKLLIYAASNVESGVPARFSGSGSGTDFSLNIHPVEEDDFAMYFCQQSRKIPYTFGGGTKLEIK

SEQ ID NO: 44 - DNA, 333 bp, Artificial Sequence
  3B8VL nucleotide
gatatcgtgctgacccaatctccagcttctttggctgtgtctctagggcagagagccaccatctcctgcagagccagtgaaagtgttgaatattatggcacaagtttaatgcagtggtaccaacagaaaccaggacagccacccaaactcctcatctatgctgcatccaacgtagaatctggggtccctgccaggtttagtggcagtgggtctgggacagacttcagcctcaacatccatcctgtggaggaggatgattttgcaatgtatttctgtcagcaaagtaggaagattccttacacgttcggaggggggaccaagctggaaataaaa

SEQ ID NO: 45 - protein, 5 aa, Artificial Sequence
  3B8 HCDR1
NYAVS

SEQ ID NO: 46 - protein, 14 aa, Artificial Sequence
  3B8 HCDR2
WGDGTTNYHSALIS

SEQ ID NO: 47 - protein, 13 aa, Artificial Sequence
  3B8 HCDR3
EGDYGDYVGWFAY

SEQ ID NO: 48 - protein, 15 aa, Artificial Sequence
  3B8 LCDR1
RASESVEYYGTSLMQ

SEQ ID NO: 49 - protein, 7 aa, Artificial Sequence
  3B8 LCDR2
AASNVES

SEQ ID NO: 50 - protein, 9 aa, Artificial Sequence
  3B8 LCDR3
QQSRKIPYT

SEQ ID NO: 51 - protein, 123 aa, Artificial Sequence
  4G1 VH
QVQLQQSGPELVKPGASVKISCKASGYSFTAYNMNWVKQSKGKSLEWIGLINPNYATTSYNQKFKDKATLTVDQSSSTAYMQLNSLTSEDSAVYYCAYYSYYSYGGGYAMDYWGQGTSVTVSS

SEQ ID NO: 52 - DNA, 369 bp, Artificial Sequence
  4G1 VH nucleotide
caggtccagctgcagcagtccggacctgagctggtgaagcctggcgcttcagtgaagatatcatgcaaggcttctggttactcattcactgcctacaacatgaactgggtgaagcagagcaagggaaagagccttgagtggattggactaattaatcctaactatgccacgactagttacaatcagaagttcaaggacaaggccacattgactgtggaccaatcttccagcacagcctacatgcagctcaacagcctgacatctgaggactctgcagtctattactgtgcctactatagttactatagttacggggggggatatgctatggactactggggtcaaggaacctcagtcaccgtctcctca

SEQ ID NO: 53 - protein, 107 aa, Artificial Sequence
  4G1VL
DILLTQSPAILSVSPGERVSFSCRASQSIGTSIHWYQQRTNGSPRLLIKYASESISGIPSRFSGSGSGTDFILSINSVESEDIADYYCQQSNSWPWTFGGGTRLEIK

SEQ ID NO: 54 - DNA, 321 bp, Artificial Sequence
  4G1VL nucleotide
gatatcttgctgacccaatctccagccatcctgtctgtgagtccaggagaaagagtcagtttttcctgcagggccagtcagagcattggcacaagcatacactggtatcagcaaagaacaaatgggtctccaaggcttctcataaagtatgcttctgagtctatctctgggatcccttccaggtttagtggcagtggatcagggacagattttattcttagcatcaacagtgtggagtctgaggatattgctgattattactgtcagcaaagtaatagctggccgtggacgttcggtggaggcaccaggctggaaatcaaa

SEQ ID NO: 55 - protein, 5 aa, Artificial Sequence
  4G1 HCDR1
AYNMN

SEQ ID NO: 56 - protein, 17 aa, Artificial Sequence
  4G1 HCDR2
LINPNYATTSYNQKFKD

SEQ ID NO: 57 - protein, 14 aa, Artificial Sequence
  4G1 HCDR3
YSYYSYGGGYAMDY

SEQ ID NO: 58 - protein, 11 aa, Artificial Sequence
  4G1 LCDR1
RASQSIGTSIH

SEQ ID NO: 59 - protein, 7 aa, Artificial Sequence
  4G1 LCDR2
YASESIS

SEQ ID NO: 60 - protein, 9 aa, Artificial Sequence
  4G1 LCDR3
QQSNSWPWT

SEQ ID NO: 61 - protein, 121 aa, Artificial Sequence
  4H3 VH
QVQLQQSGPELVKPGASVKISCKASGYSFTAYNINWVKQTNGKSLEWIGIINPNYGTTSYNQKFKGKATLTVDQSSSTAYMQLNSLTSEDSAVYYCARRNGDYVGYAMDSWGQGTSVTVSS

SEQ ID NO: 62 - DNA, 363 bp, Artificial Sequence
  4H3 VH nucleotide
caggtgcagctgcagcagtctggacctgagctggtgaagcctggcgcttcagtgaagatatcctgcaaggcttctggttactcattcactgcctacaacattaactgggtgaagcagaccaatggaaagagccttgagtggattggaataattaatcctaactatggtactactagttacaaccagaagttcaagggcaaggccacattgactgtagaccaatcttccagtacagcctacatgcagctcaacagcctgacatctgaggactctgcagtctattactgtgcaagacggaatggtgactacgtgggatatgctatggactcctggggtcaaggaacctcagtcaccgtctcctca

SEQ ID NO: 63 - protein, 107 aa, Artificial Sequence
  4H3VL
DIVLTQSPAILSVSPGERVSFSCRASQSIGTSMHWYQQRKNGSPRLLIKYASESISGIPSRFSGSGSGTDFTLSINSVESEDIADYYCQQTNNWPWTFGGGTKLEFK

SEQ ID NO: 64 - DNA, 321 bp, Artificial Sequence
  4H3VL nucleotide
gatatcgttctcacccagtctccagccatcctctctgtgagtccaggagaaagagtcagtttctcctgcagggccagtcagagcattggcacaagcatgcactggtatcagcaaagaaaaaatggttctccaaggcttctcataaagtatgcttctgagtctatctctgggatcccttccaggtttagtggcagtggatcagggacagattttactcttagcatcaacagtgtggagtctgaggatattgcagattattactgtcaacaaactaataactggccgtggacgttcggtggaggcaccaagctggaattcaaa

SEQ ID NO: 65 - protein, 5 aa, Artificial Sequence
  4H3 HCDR1
AYNIN

SEQ ID NO: 66 - protein, 17 aa, Artificial Sequence
  4H3 HCDR2
IINPNYGTTSYNQKFKG

SEQ ID NO: 67 - protein, 12 aa, Artificial Sequence
  4H3 HCDR3
RNGDYVGYAMDS

SEQ ID NO: 68 - protein, 11 aa, Artificial Sequence
  4H3 LCDR1
RASQSIGTSMH

SEQ ID NO: 69 - protein, 7 aa, Artificial Sequence
  4H3 LCDR2
YASESIS

SEQ ID NO: 70 - protein, 9 aa, Artificial Sequence
  4H3 LCDR3
QQTNNWPWT

SEQ ID NO: 71 - protein, 117 aa, Artificial Sequence
  2G3 VH
EVKLQESGGGLVKPGGSLKLSCAASGFTFSSFAMSWIRQTPEKRLEWVAAISDGGTYTYYPNNVKGRFTISRDDAKNNLYLQMSHLKSEDTAMYYCVRNRGGPFDYWGQGTTLTVSS

SEQ ID NO: 72 - DNA, 351 bp, Artificial Sequence
  2G3 VH nucleotide
gaggtgaagctgcaggagtctgggggaggcttagtgaagcctggagggtccctgaaactctcctgtgcagcctctggattcactttcagtagctttgccatgtcttggattcgccagactccggaaaagaggctggagtgggtcgcggccattagtgatggtggtacttacacctactatccaaacaatgtaaagggccgattcaccatctccagagacgatgccaagaataacctgtacctgcaaatgagtcatctgaagtctgaggacacagccatgtattactgtgtaagaaatagggggggaccctttgactactggggccaaggcaccactctcacagtctcctca

SEQ ID NO: 73 - protein, 106 aa, Artificial Sequence
  2G3VL
DIVLTQSPAIMSASPGEKVTMTCSASSSVSYMNWYQQKSGTSPKRWIYDTSKLASGVPVRFSGSGSGTSYSLTISSMEAEDAATYYCQQWNSNPPTFGAGTKLELK

SEQ ID NO: 74 - DNA, 318 bp, Artificial Sequence
  2G3VL nucleotide
gatatcgtgctcactcagtctccagcaatcatgtctgcatctccaggggagaaggtcaccatgacctgcagtgccagctcaagtgtaagttacatgaactggtaccagcagaagtcaggcacctcccccaaaagatggatttatgacacatccaaactggcttctggagtccctgttcgcttcagtggcagtgggtctgggacctcttactctctcacaatcagcagcatggaggctgaagatgctgccacttattactgccagcagtggaatagtaacccacccacgttcggtgctgggaccaagctggagctgaaa

SEQ ID NO: 75 - protein, 5 aa, Artificial Sequence
  2G3 HCDR1
SFAMS

SEQ ID NO: 76 - protein, 17 aa, Artificial Sequence
  2G3 HCDR2
AISDGGTYTYYPNNVKG

SEQ ID NO: 77 - protein, 8 aa, Artificial Sequence
  2G3 HCDR3
NRGGPFDY

SEQ ID NO: 78 - protein, 10 aa, Artificial Sequence
  2G3 LCDR1
SASSSVSYMN

SEQ ID NO: 79 - protein, 7 aa, Artificial Sequence
  2G3 LCDR2
DTSKLAS

SEQ ID NO: 80 - protein, 9 aa, Artificial Sequence
  2G3 LCDR3
QQWNSNPPT

SEQ ID NO: 81 - protein, 117 aa, Artificial Sequence
  2F11 VH
EVQLQESGGDLVKPGGSLKLSCAASGFTFSSYAMSWVRQTPEKRLEWVAIIGDGDTYTYYPDSVKGRFTVSRDNAKNNLYLQMSHLKSEDTAMYYCVRTRGGPFDYWGQGTTLTVSS

SEQ ID NO: 82 - DNA, 351 bp, Artificial Sequence
  2F11 VH nucleotide
gaggtgcagctgcaggagtctgggggagacttagtgaagcctggagggtccctgaaactctcctgtgcagcctctggattcactttcagtagctatgccatgtcttgggttcgccagactccggaaaagaggctggagtgggtcgcaatcattggtgatggtgatacttacacctactatccagacagtgtaaagggccgattcaccgtctccagagacaatgccaagaacaacctctacctgcaaatgagccatctgaagtctgaggacacagccatgtattactgtgtaagaactagggggggaccctttgactactggggccaaggcaccactctcacagtctcctca

SEQ ID NO: 83 - protein, 106 aa, Artificial Sequence
  2F11VL
DIVLTQTPALMSASPGEKVTMTCSASSSVGSMHWYQQKSGTSPKRWIYDTSKLASGVPARFSGSGSGTSYSLTISSMEAEDAATYYCQQWSSIPPTFGAGTTLELK

SEQ ID NO: 84 - DNA, 318 bp, Artificial Sequence
  2F11VL nucleotide
gatatcgtgctcacccaaactccagcactcatgtctgcatctccaggggagaaggtcaccatgacctgcagtgccagctcaagtgtaggttccatgcactggtaccagcagaagtcaggcacctcccccaaaagatggatttatgacacatccaaactggcttctggagtccctgctcgcttcagtggcagtgggtctgggacctcttactctctcacaatcagcagcatggaggctgaagatgctgccacttattactgccaacagtggagtagtatcccacccacgttcggtgctgggaccacgctggagctgaaa

SEQ ID NO: 85 - protein, 5 aa, Artificial Sequence
  2F11 HCDR1
SYAMS

SEQ ID NO: 86 - protein, 17 aa, Artificial Sequence
  2F11 HCDR2
IIGDGDTYTYYPDSVKG

SEQ ID NO: 87 - protein, 8 aa, Artificial Sequence
  2F11 HCDR3
TRGGPFDY

SEQ ID NO: 88 - protein, 10 aa, Artificial Sequence
  2F11 LCDR1
SASSSVGSMH

SEQ ID NO: 89 - protein, 7 aa, Artificial Sequence
  2F11 LCDR2
DTSKLAS

SEQ ID NO: 90 - protein, 9 aa, Artificial Sequence
  2F11 LCDR3
QQWSSIPPT

SEQ ID NO: 91 - protein, 106 aa, Artificial Sequence
  16647VL
EILLTQSPAFMSATPGEKVTITCSASSSVGSMHWYQQKSGQSPRRLIYDTSKLASGVPDRFSGSGSGTDYTLTISSLEAEDAATYYCQQWSSIPPTFGAGTTLELK

SEQ ID NO: 92 - DNA, 318 bp, Artificial Sequence
  16647VL nucleotide
gagatcctgctgacccagagccctgcctttatgagcgccacccccggcgagaaggtgaccatcacctgcagcgccagcagcagcgtgggcagcatgcactggtatcaacagaagagcggccagagccccaggaggctgatctacgacaccagcaagctggccagcggcgtgcctgacaggttctctggtagcggcagcggcaccgactacaccctgaccatcagcagcctggaggccgaagacgccgccacctactactgccagcagtggagcagcatccctcccaccttcggcgctggaaccaccctggagctgaag

SEQ ID NO: 93 - protein, 117 aa, Artificial Sequence
  9419VH
EVHLQESGGALVKPGGSLRLSCAASGFTFSSYAMSWVRQAPEKGLEWVAIIGDGDTYTYYPDSVKGRFTISRDNAKNTLYLQMSNLKSEDTAMYYCVRTRGGPFDYWGQGTTLTVSS

SEQ ID NO: 94 - DNA, 351 bp, Artificial Sequence
  9419VH nucleotide
gaggtgcacctgcaggagtctggtggagccctggtgaagcccggaggaagcctgagactgagctgcgccgccagcggcttcaccttcagcagctacgccatgagctgggtgagacaggcccctgagaagggcctggagtgggtggccatcatcggcgacggcgacacctacacctactaccccgacagcgtgaagggcaggttcaccatcagcagggacaacgctaagaacaccctgtacctgcagatgagcaacctgaagagcgaggacaccgccatgtactactgcgtgaggaccagaggcggccctttcgactactggggccagggcaccaccctgacagtgagcagc

SEQ ID NO: 95 - protein, 117 aa, Artificial Sequence
  d9419VH
EVHLQESGGALVKPGGSLRLSCAASGFTFSSYAMSWVRQKPEKNLEWVAIIGDGDTYTYYPDSVKGRFTISRDNAKNTLYLQMSDLKSEDTAMYYCVRTRGGPFDYWGQGTTLTVSS

SEQ ID NO: 96 - DNA, 351 bp, Artificial Sequence
  d9419VH nucleotide
gaggtgcatctgcaggagagcggcggagccctggtgaaacctggcggaagcctgagactgagctgcgccgcctccggcttcaccttcagctcctacgccatgagctgggtgaggcagaagcccgagaagaacctggagtgggtggccatcatcggcgacggcgacacctacacctactaccccgacagcgtgaagggcaggttcaccatcagcagggacaacgccaagaacaccctgtacctgcagatgagcgacctgaagagcgaggacaccgccatgtactactgcgtgaggaccaggggcggccctttcgactattggggccagggcacaaccctgaccgtgagcagc

SEQ ID NO: 97 - protein, 117 aa, Artificial Sequence
  9424VH
EVHLQESGGGLVKPGGSLRLSCAASGFTFSSYAMSWVRQTPEKGLEWVAIIGDGDTYTYYPDSVKGRFTISRDNAKNTLYLQMNSLKSEDTAMYYCVRTRGGPFDYWGQGTTLTVSS

SEQ ID NO: 98 - DNA, 351 bp, Artificial Sequence
  9424VH nucleotide
gaggtgcacctgcaggagtctggtggaggcctggtgaagcccggaggaagcctgagactgagctgcgccgccagcggcttcaccttcagcagctacgccatgagctgggtgagacagacccctgagaagggcctggagtgggtggccatcatcggcgacggcgacacctacacctactaccccgacagcgtgaagggcaggttcaccatcagcagggacaacgctaagaacaccctgtacctgcagatgaacagcctgaagagcgaggacaccgccatgtactactgcgtgaggaccagaggcggccctttcgactactggggccagggcaccaccctgacagtgagcagc

SEQ ID NO: 99 - protein, 117 aa, Artificial Sequence
  d9424VH
EVHLQESGGGLVKPGGSLRLSCAASGFTFSSYAMSWVRQTPEKNLEWVAIIGDGDTYTYYPDSVKGRFTISRDNAKNTLYLQMNDLKSEDTAMYYCVRTRGGPFDYWGQGTTLTVSS

SEQ ID NO: 100 - DNA, 351 bp, Artificial Sequence
  d9424 nucleotide
gaggtgcatctgcaggagagcggcggaggcctggtgaaacctggcggaagcctgagactgagctgcgccgcctccggcttcaccttcagctcctacgccatgagctgggtgaggcagacgcccgagaagaacctggagtgggtggccatcatcggcgacggcgacacctacacctactaccccgacagcgtgaagggcaggttcaccatcagcagggacaacgccaagaacaccctgtacctgcagatgaacgacctgaagagcgaggacaccgccatgtactactgcgtgaggaccaggggcggccctttcgactattggggccagggcacaaccctgaccgtgagcagc

SEQ ID NO: 101 - protein, 117 aa, Artificial Sequence
  12674VH
EVHLQESGGGLVKPGGSLRLSCAASGFTFSSYAMSWVRQAPGKGLEWVAIIGDGDTYTYYPDSVKGRFTISRDNSKNRLYLQMNSLKSEDTAMYYCVRTRGGPFDYWGQGTTLTVSS

SEQ ID NO: 102 - DNA, 351 bp, Artificial Sequence
  12674VH nucleotide
gaggtgcacctgcaagagagcggaggaggcctggtgaaacctggcggcagcctgaggctgagctgtgctgccagcggcttcaccttctccagctacgccatgagctgggtgaggcaggcgcccggcaaaggcctggagtgggtggccatcatcggcgacggcgacacctacacctactaccccgacagcgtgaagggcaggttcaccatcagcagggacaacagcaagaacaggctgtacctgcagatgaacagcctgaagagcgaggacaccgccatgtactactgcgtgaggaccagaggcggccctttcgactactggggccagggaaccaccctgaccgtgagcagc

SEQ ID NO: 103 - protein, 117 aa, Artificial Sequence
  d12674VH
EVHLQESGGGLVKPGGSLRLSCAASGFTFSSYAMSWVRQAPGKGLEWVAIIGDGDTYTYYPDSVKGRFTISRDNSKNRLYLQMNDLKSEDTAMYYCVRTRGGPFDYWGQGTTLTVSS

SEQ ID NO: 104 - DNA, 351 bp, Artificial Sequence
  d12674 nucleotide
gaggtgcacctgcaagagagcggaggcggactggtgaaacctggcggcagcctgagactgagctgtgccgccagcggcttcaccttcagcagctacgccatgagctgggtgaggcaggcccccggtaagggcctggagtgggtggccatcatcggcgacggcgacacctacacctactaccccgacagcgtgaagggcagattcaccatcagcagggacaactccaagaacaggctgtacctgcagatgaacgacctgaagagcgaggacaccgccatgtactactgcgtgaggaccaggggcggccctttcgattactggggccagggcacaaccctgaccgtgagcagc

SEQ ID NO: 105 - protein, 117 aa, Artificial Sequence
  12996VH
EVHLQESGGGLVKPGGSLRLSCAASGFTFSSYAMSWVRQAPEKGLEWVAIIGDGDTYTYYPDSVKGRFTISRDNSKNRLYLQMNSLKSEDTAMYYCVRTRGGPFDYWGQGTTLTVSS

SEQ ID NO: 106 - DNA, 351 bp, Artificial Sequence
  12996VH nucleotide
gaggtgcacctgcaagagagcggaggaggcctggtgaaacctggcggcagcctgaggctgagctgtgctgccagcggcttcaccttctccagctacgccatgagctgggtgaggcaggcgcccgagaaaggcctggagtgggtggccatcatcggcgacggcgacacctacacctactaccccgacagcgtgaagggcaggttcaccatcagcagggacaacagcaagaacaggctgtacctgcagatgaacagcctgaagagcgaggacaccgccatgtactactgcgtgaggaccagaggcggccctttcgactactggggccagggaaccaccctgaccgtgagcagc

SEQ ID NO: 107 - protein, 117 aa, Artificial Sequence
  d12996VH
EVHLQESGGGLVKPGGSLRLSCAASGFTFSSYAMSWVRQEPEKNLEWVAIIGDGDTYTYYPDSVKGRFTISRDNSKNRLYLQMNDLKSEDTAMYYCVRTRGGPFDYWGQGTTLTVSS

SEQ ID NO: 108 - DNA, 351 bp, Artificial Sequence
  d12996VH nucleotide
gaggtgcacctgcaagagagcggaggcggactggtgaaacctggcggcagcctgagactgagctgtgccgccagcggcttcaccttcagcagctacgccatgagctgggtgaggcaggaacccgagaagaacctggagtgggtggccatcatcggcgacggcgacacctacacctactaccccgacagcgtgaagggcagattcaccatcagcagggacaactccaagaacaggctgtacctgcagatgaacgacctgaagagcgaggacaccgccatgtactactgcgtgaggaccaggggcggccctttcgattactggggccagggcacaaccctgaccgtgagcagc

SEQ ID NO: 109 - protein, 117 aa, Artificial Sequence
  14822VH
EVHLQESGGGLVKPGGSLRLSCAASGFTFSSYAMSWVRQMPGKGLEWVAIIGDGDTYTYYPDSVKGRFTISRDNSKNTLYLQMNSLKSEDTAMYYCVRTRGGPFDYWGQGTTLTVSS

SEQ ID NO: 110 - DNA, 351 bp, Artificial Sequence
  14822VH nucleotide
gaggtgcacctgcaagagagcggaggaggcctggtgaaacctggcggcagcctgaggctgagctgtgctgccagcggcttcaccttctccagctacgccatgagctgggtgaggcagatgcccggcaaaggcctggagtgggtggccatcatcggcgacggcgacacctacacctactaccccgacagcgtgaagggcaggttcaccatcagcagggacaacagcaagaacacgctgtacctgcagatgaacagcctgaagagcgaggacaccgccatgtactactgcgtgaggaccagaggcggccctttcgactactggggccagggaaccaccctgaccgtgagcagc

SEQ ID NO: 111 - protein, 117 aa, Artificial Sequence
  d14882VH
EVHLQESGGGLVKPGGSLRLSCAASGFTFSSYAMSWVRQTPDKGLEWVAIIGDGDTYTYYPDSVKGRFTISRDNSKNTLYLQMNDLKSEDTAMYYCVRTRGGPFDYWGQGTTLTVSS

SEQ ID NO: 112 - DNA, 351 bp, Artificial Sequence
  d14882VH nucleotide
gaggtgcacctgcaagagagcggaggcggactggtgaaacctggcggcagcctgagactgagctgtgccgccagcggcttcaccttcagcagctacgccatgagctgggtgaggcagacccccgataagggcctggagtgggtggccatcatcggcgacggcgacacctacacctactaccccgacagcgtgaagggcagattcaccatcagcagggacaactccaagaacacgctgtacctgcagatgaacgacctgaagagcgaggacaccgccatgtactactgcgtgaggaccaggggcggccctttcgattactggggccagggcacaaccctgaccgtgagcagc

SEQ ID NO: 113 - protein, 117 aa, Artificial Sequence
  16647VH
QVELRESGGGLVKPGGSLRLSCAASGFTFSSYAMSWVRQMPGKGLEWVAIIGDGDTYTYYPDSVKGRFTISRDNSKNRLYLQMNSLKSEDTAMYYCVRTRGGPFDYWGQGTTLTVSS

SEQ ID NO: 114 - DNA, 351 bp, Artificial Sequence
  16647VH nucleotide
caggtggagctgagagagagcggaggaggcctggtgaaacctggcggcagcctgaggctgagctgtgctgccagcggcttcaccttctccagctacgccatgagctgggtgaggcagatgcccggcaaaggcctggagtgggtggccatcatcggcgacggcgacacctacacctactaccccgacagcgtgaagggcaggttcaccatcagcagggacaacagcaagaacaggctgtacctgcagatgaacagcctgaagagcgaggacaccgccatgtactactgcgtgaggaccagaggcggccctttcgactactggggccagggaaccaccctgaccgtgagcagc

SEQ ID NO: 115 - protein, 117 aa, Artificial Sequence
  d16647VH
QVELRESGGGLVKPGGSLRLSCAASGFTFSSYAMSWVRQTPDKGLEWVAIIGDGDTYTYYPDSVKGRFTISRDNSKNRLYLQMNDLKSEDTAMYYCVRTRGGPFDYWGQGTTLTVSS

SEQ ID NO: 116 - DNA, 351 bp, Artificial Sequence
  d16647VH nucleotide
caggtggagctgagggagagcggaggcggactggtgaaacctggcggcagcctgagactgagctgtgccgccagcggcttcaccttcagcagctacgccatgagctgggtgaggcagacccccgataagggcctggagtgggtggccatcatcggcgacggcgacacctacacctactaccccgacagcgtgaagggcagattcaccatcagcagggacaactccaagaacaggctgtacctgcagatgaacgacctgaagagcgaggacaccgccatgtactactgcgtgaggaccaggggcggccctttcgattactggggccagggcacaaccctgaccgtgagcagc

SEQ ID NO: 117 - protein, 214 aa, Artificial Sequence
  m2E7light chain
DIVMTQSTAIMSASPGEKVTMTCSASSSVSYMHWYQQKSGTSPRRWIYDTSRLASGVPARFSGSGSGTSYSLTISSMEAEDAATYYCQQWSNTPPFTFGAGTKLELKRTVAAPSVFIFPPSDEQLKSGTASVVCLLNNFYPREAKVQWKVDNALQSGNSQESVTEQDSKDSTYSLSSTLTLSKADYEKHKVYACEVTHQGLSSPVTKSFNRGEC

SEQ ID NO: 118 - protein, 446 aa, Artificial Sequence
  m2E7 heavy chain
EVQLQESGPELKKPGETVKISCKASGYTFTTYGMSWVKQAPGKGLQWMGWINTNSGVPTYVEDFKGRFAFSLESSANTAYLQINNLKNEDTAIYFCTREGDALDYWGQGTSVTVSSASTKGPSVFPLAPSSKSTSGGTAALGCLVKDYFPEPVTVSWNSGALTSGVHTFPAVLQSSGLYSLSSVVTVPSSSLGTQTYICNVNHKPSNTKVDKKVEPKSCDKTHTCPPCPAPELLGGPSVFLFPPKPKDTLMISRTPEVTCVVVDVSHEDPEVKFNWYVDGVEVHNAKTKPREEQYNSTYRVVSVLTVLHQDWLNGKEYKCKVSNKALPAPIEKTISKAKGQPREPQVYTLPPSRDELTKNQVSLTCLVKGFYPSDIAVEWESNGQPENNYKTTPPVLDSDGSFFLYSKLTVDKSRWQQGNVFSCSVMHEALHNHYTQKSLSLSPGK

SEQ ID NO: 119 - protein, 214 aa, Artificial Sequence
  m2B8 light chain
DIVMTQSPSYLAASPGETITINCRASKSISKYLAWYREKPGKTNNLLIYSGSTLQSGIPSRFSGSGSGTDFTLTISSLEPEDFAMYYCQQHNEYPLTFGAGTKLELKRTVAAPSVFIFPPSDEQLKSGTASVVCLLNNFYPREAKVQWKVDNALQSGNSQESVTEQDSKDSTYSLSSTLTLSKADYEKHKVYACEVTHQGLSSPVTKSFNRGEC

SEQ ID NO: 120 - protein, 450 aa, Artificial Sequence
  m2B8 heavy chain
EVQLQESGGGLVQPKGSLKLSCAASGFNFNTYTMNWVRQAPGKGLEWVARIRYKSNNYATYYADSVKDRFTISRDDSESILYLQMNNLRTDDTAIYFCVRELGLWYFDVWGAGTTVTVSSASTKGPSVFPLAPSSKSTSGGTAALGCLVKDYFPEPVTVSWNSGALTSGVHTFPAVLQSSGLYSLSSVVTVPSSSLGTQTYICNVNHKPSNTKVDKKVEPKSCDKTHTCPPCPAPELLGGPSVFLFPPKPKDTLMISRTPEVTCVVVDVSHEDPEVKFNWYVDGVEVHNAKTKPREEQYNSTYRVVSVLTVLHQDWLNGKEYKCKVSNKALPAPIEKTISKAKGQPREPQVYTLPPSRDELTKNQVSLTCLVKGFYPSDIAVEWESNGQPENNYKTTPPVLDSDGSFFLYSKLTVDKSRWQQGNVFSCSVMHEALHNHYTQKSLSLSPGK

SEQ ID NO: 121 - protein, 214 aa, Artificial Sequence
  m4H3 light chain
DIVLTQSPAILSVSPGERVSFSCRASQSIGTSMHWYQQRKNGSPRLLIKYASESISGIPSRFSGSGSGTDFTLSINSVESEDIADYYCQQTNNWPWTFGGGTKLEFKRTVAAPSVFIFPPSDEQLKSGTASVVCLLNNFYPREAKVQWKVDNALQSGNSQESVTEQDSKDSTYSLSSTLTLSKADYEKHKVYACEVTHQGLSSPVTKSFNRGEC

SEQ ID NO: 122 - protein, 451 aa, Artificial Sequence
  m4H3 heavy chain
QVQLQQSGPELVKPGASVKISCKASGYSFTAYNINWVKQTNGKSLEWIGIINPNYGTTSYNQKFKGKATLTVDQSSSTAYMQLNSLTSEDSAVYYCARRNGDYVGYAMDSWGQGTSVTVSSASTKGPSVFPLAPSSKSTSGGTAALGCLVKDYFPEPVTVSWNSGALTSGVHTFPAVLQSSGLYSLSSVVTVPSSSLGTQTYICNVNHKPSNTKVDKKVEPKSCDKTHTCPPCPAPELLGGPSVFLFPPKPKDTLMISRTPEVTCVVVDVSHEDPEVKFNWYVDGVEVHNAKTKPREEQYNSTYRVVSVLTVLHQDWLNGKEYKCKVSNKALPAPIEKTISKAKGQPREPQVYTLPPSRDELTKNQVSLTCLVKGFYPSDIAVEWESNGQPENNYKTTPPVLDSDGSFFLYSKLTVDKSRWQQGNVFSCSVMHEALHNHYTQKSLSLSPGK

SEQ ID NO: 123 - protein, 214 aa, Artificial Sequence
  m3E7 light chain
DIVMTQTTAIMSAFPGEKVTMTCSASSSVSYMHWYQQKSGTSPKRWIYDTSKLASGVPVRFSGSGSGTSYSLTISNMEAEDAATYYCQQWSRNPPFTFGAGTKLELKRTVAAPSVFIFPPSDEQLKSGTASVVCLLNNFYPREAKVQWKVDNALQSGNSQESVTEQDSKDSTYSLSSTLTLSKADYEKHKVYACEVTHQGLSSPVTKSFNRGEC

SEQ ID NO: 124 - protein, 446 aa, Artificial Sequence
  m3E7 heavy chain
QIQLVQSGPELKKPGETVKISCKASGYTFTTYGMSWVKQAPGKGLHWMGWINTHSGAPTYVDDFKGRFAFSLETSASTAFLQINNLINEDTATYFCAREGDALDYWGQGTSVTVSSASTKGPSVFPLAPSSKSTSGGTAALGCLVKDYFPEPVTVSWNSGALTSGVHTFPAVLQSSGLYSLSSVVTVPSSSLGTQTYICNVNHKPSNTKVDKKVEPKSCDKTHTCPPCPAPELLGGPSVFLFPPKPKDTLMISRTPEVTCVVVDVSHEDPEVKFNWYVDGVEVHNAKTKPREEQYNSTYRVVSVLTVLHQDWLNGKEYKCKVSNKALPAPIEKTISKAKGQPREPQVYTLPPSRDELTKNQVSLTCLVKGFYPSDIAVEWESNGQPENNYKTTPPVLDSDGSFFLYSKLTVDKSRWQQGNVFSCSVMHEALHNHYTQKSLSLSPGK

SEQ ID NO: 125 - protein, 214 aa, Artificial Sequence
  m1A8 light chain
DIVLTQSPAILSVSPGERVSFSCRASQSIGTSIHWYQQRTNGSPRLLIKYASESISGIPSRFSGSGSGTDFTLSINSVESEDIADYYCQQSNSWPLTFGAGTKLELKRTVAAPSVFIFPPSDEQLKSGTASVVCLLNNFYPREAKVQWKVDNALQSGNSQESVTEQDSKDSTYSLSSTLTLSKADYEKHKVYACEVTHQGLSSPVTKSFNRGEC

SEQ ID NO: 126 - protein, 452 aa, Artificial Sequence
  m1A8 heavy chain
EVQLQESGAELVKPGASVKLSCKASGYSFTSSWMHWVKQRPGQGLEWIGMIHPDSGFTNYNEKFKSKATLTVDKSSSTAYMRLSSLTSEDSAVYYCARTSYYDTSYTSMDFWGQGNSVTVSSASTKGPSVFPLAPSSKSTSGGTAALGCLVKDYFPEPVTVSWNSGALTSGVHTFPAVLQSSGLYSLSSVVTVPSSSLGTQTYICNVNHKPSNTKVDKKVEPKSCDKTHTCPPCPAPELLGGPSVFLFPPKPKDTLMISRTPEVTCVVVDVSHEDPEVKFNWYVDGVEVHNAKTKPREEQYNSTYRVVSVLTVLHQDWLNGKEYKCKVSNKALPAPIEKTISKAKGQPREPQVYTLPPSRDELTKNQVSLTCLVKGFYPSDIAVEWESNGQPENNYKTTPPVLDSDGSFFLYSKLTVDKSRWQQGNVFSCSVMHEALHNHYTQKSLSLSPGK

SEQ ID NO: 127 - protein, 214 aa, Artificial Sequence
  m4G1 light chain
DILLTQSPAILSVSPGERVSFSCRASQSIGTSIHWYQQRTNGSPRLLIKYASESISGIPSRFSGSGSGTDFILSINSVESEDIADYYCQQSNSWPWTFGGGTRLEIKRTVAAPSVFIFPPSDEQLKSGTASVVCLLNNFYPREAKVQWKVDNALQSGNSQESVTEQDSKDSTYSLSSTLTLSKADYEKHKVYACEVTHQGLSSPVTKSFNRGEC

SEQ ID NO: 128 - protein, 453 aa, Artificial Sequence
  m4G1 heavy chain
QVQLQQSGPELVKPGASVKISCKASGYSFTAYNMNWVKQSKGKSLEWIGLINPNYATTSYNQKFKDKATLTVDQSSSTAYMQLNSLTSEDSAVYYCAYYSYYSYGGGYAMDYWGQGTSVTVSSASTKGPSVFPLAPSSKSTSGGTAALGCLVKDYFPEPVTVSWNSGALTSGVHTFPAVLQSSGLYSLSSVVTVPSSSLGTQTYICNVNHKPSNTKVDKKVEPKSCDKTHTCPPCPAPELLGGPSVFLFPPKPKDTLMISRTPEVTCVVVDVSHEDPEVKFNWYVDGVEVHNAKTKPREEQYNSTYRVVSVLTVLHQDWLNGKEYKCKVSNKALPAPIEKTISKAKGQPREPQVYTLPPSRDELTKNQVSLTCLVKGFYPSDIAVEWESNGQPENNYKTTPPVLDSDGSFFLYSKLTVDKSRWQQGNVFSCSVMHEALHNHYTQKSLSLSPGK

SEQ ID NO: 129 - protein, 213 aa, Artificial Sequence
  m2G3 light chain
DIVLTQSPAIMSASPGEKVTMTCSASSSVSYMNWYQQKSGTSPKRWIYDTSKLASGVPVRFSGSGSGTSYSLTISSMEAEDAATYYCQQWNSNPPTFGAGTKLELKRTVAAPSVFIFPPSDEQLKSGTASVVCLLNNFYPREAKVQWKVDNALQSGNSQESVTEQDSKDSTYSLSSTLTLSKADYEKHKVYACEVTHQGLSSPVTKSFNRGEC

SEQ ID NO: 130 - protein, 447 aa, Artificial Sequence
  m2G3 heavy chain
EVKLQESGGGLVKPGGSLKLSCAASGFTFSSFAMSWIRQTPEKRLEWVAAISDGGTYTYYPNNVKGRFTISRDDAKNNLYLQMSHLKSEDTAMYYCVRNRGGPFDYWGQGTTLTVSSASTKGPSVFPLAPSSKSTSGGTAALGCLVKDYFPEPVTVSWNSGALTSGVHTFPAVLQSSGLYSLSSVVTVPSSSLGTQTYICNVNHKPSNTKVDKKVEPKSCDKTHTCPPCPAPELLGGPSVFLFPPKPKDTLMISRTPEVTCVVVDVSHEDPEVKFNWYVDGVEVHNAKTKPREEQYNSTYRVVSVLTVLHQDWLNGKEYKCKVSNKALPAPIEKTISKAKGQPREPQVYTLPPSRDELTKNQVSLTCLVKGFYPSDIAVEWESNGQPENNYKTTPPVLDSDGSFFLYSKLTVDKSRWQQGNVFSCSVMHEALHNHYTQKSLSLSPGK

SEQ ID NO: 131 - protein, 213 aa, Artificial Sequence
  m2F11 light chain
DIVLTQTPALMSASPGEKVTMTCSASSSVGSMHWYQQKSGTSPKRWIYDTSKLASGVPARFSGSGSGTSYSLTISSMEAEDAATYYCQQWSSIPPTFGAGTTLELKRTVAAPSVFIFPPSDEQLKSGTASVVCLLNNFYPREAKVQWKVDNALQSGNSQESVTEQDSKDSTYSLSSTLTLSKADYEKHKVYACEVTHQGLSSPVTKSFNRGEC

SEQ ID NO: 132 - protein, 447 aa, Artificial Sequence
  m2F11 heavy chain
EVQLQESGGDLVKPGGSLKLSCAASGFTFSSYAMSWVRQTPEKRLEWVAIIGDGDTYTYYPDSVKGRFTVSRDNAKNNLYLQMSHLKSEDTAMYYCVRTRGGPFDYWGQGTTLTVSSASTKGPSVFPLAPSSKSTSGGTAALGCLVKDYFPEPVTVSWNSGALTSGVHTFPAVLQSSGLYSLSSVVTVPSSSLGTQTYICNVNHKPSNTKVDKKVEPKSCDKTHTCPPCPAPELLGGPSVFLFPPKPKDTLMISRTPEVTCVVVDVSHEDPEVKFNWYVDGVEVHNAKTKPREEQYNSTYRVVSVLTVLHQDWLNGKEYKCKVSNKALPAPIEKTISKAKGQPREPQVYTLPPSRDELTKNQVSLTCLVKGFYPSDIAVEWESNGQPENNYKTTPPVLDSDGSFFLYSKLTVDKSRWQQGNVFSCSVMHEALHNHYTQKSLSLSPGK

SEQ ID NO: 133 - protein, 218 aa, Artificial Sequence
  m3B8 light chain
DIVLTQSPASLAVSLGQRATISCRASESVEYYGTSLMQWYQQKPGQPPKLLIYAASNVESGVPARFSGSGSGTDFSLNIHPVEEDDFAMYFCQQSRKIPYTFGGGTKLEIKRTVAAPSVFIFPPSDEQLKSGTASVVCLLNNFYPREAKVQWKVDNALQSGNSQESVTEQDSKDSTYSLSSTLTLSKADYEKHKVYACEVTHQGLSSPVTKSFNRGEC

SEQ ID NO: 134 - protein, 451 aa, Artificial Sequence
  m3B8 heavy chain
QVQLQESGPGLVAPSQSLSITCTVSGFSLTNYAVSWVRQPPGKGLEWLGVIWGDGTTNYHSALISRLIISKDNSKSQVFLKLNSLQTDDTATYYCAKEGDYGDYVGWFAYWGQGTLVTVSAASTKGPSVFPLAPSSKSTSGGTAALGCLVKDYFPEPVTVSWNSGALTSGVHTFPAVLQSSGLYSLSSVVTVPSSSLGTQTYICNVNHKPSNTKVDKKVEPKSCDKTHTCPPCPAPELLGGPSVFLFPPKPKDTLMISRTPEVTCVVVDVSHEDPEVKFNWYVDGVEVHNAKTKPREEQYNSTYRVVSVLTVLHQDWLNGKEYKCKVSNKALPAPIEKTISKAKGQPREPQVYTLPPSRDELTKNQVSLTCLVKGFYPSDIAVEWESNGQPENNYKTTPPVLDSDGSFFLYSKLTVDKSRWQQGNVFSCSVMHEALHNHYTQKSLSLSPGK

SEQ ID NO: 135 - DNA, 652 bp, Artificial Sequence
  m2E7light chain(nucleotide)
gatattgtgatgacacaatctacagcaatcatgtctgcatctccaggggagaaggtcaccatgacctgcagtgccagctcaagtgtaagttacatgcactggtaccagcagaagtcaggcacctcccccagaagatggatttatgacacatccagactggcttctggagtccctgctcgcttcagtggcagtgggtctgggacctcttactctctcacaatcagcagcatggaggctgaagatgctgccacttattactgccagcagtggagtaataccccacccttcacgttcggtgctgggaccaagttggagctgaaacgtacggtggctgcaccatctgtcttcatcttcccgccatctgatgagcagttgaaatctggtaccgctagcgttgtgtgcctgctgaataacttttatccacgggaggctaaggtgcagtggaaagtggacaatgccctccagagcggaaatagccaagagtccgttaccgaacaggactctaaagactctacatactccctgtcctccacactgaccctctccaaggccgactatgagaaacacaaggtttacgcatgcgaggtcacacaccagggactctcctctcccgtgaccaagagcttcaaccggggagaatgctaatgaattc

SEQ ID NO: 136 - DNA, 1348 bp, Artificial Sequence
  m2E7 heavy chain(nucleotide)
gaggtgcagctgcaggagtctggacctgagctgaagaagcctggagagacagtcaagatctcctgcaaggcttctgggtataccttcacaacctatggaatgagctgggtgaaacaggctccaggaaagggtttacagtggatgggctggataaacaccaactctggagtgccaacctatgttgaggacttcaagggacggtttgccttctctttggaatcctctgccaacactgcctatttgcagatcaacaacctcaaaaatgaggacacggctatatacttctgtacaagagagggggatgctctggactactggggtcaaggaacctcagtcaccgtctcctcagccagcactaaggggccctctgtgtttccactcgccccttctagcaaaagcacttccggaggcactgcagcactcgggtgtctggtcaaagattatttccctgagccagtcaccgtgagctggaactctggcgccctcacctccggggttcacacctttccagccgtcctgcagtcctccggcctgtactccctgagcagcgtcgttaccgtgccatcctcttctctggggacccagacatacatctgcaatgtcaaccataagcctagcaacaccaaggtggacaaaaaggtcgagccaaagagctgcgataagacacacacctgccctccatgccccgcacctgaactcctgggcgggccttccgttttcctgtttcctcccaagcccaaggatacactgatgattagccgcacccccgaagtcacttgcgtggtggtggatgtgagccatgaagatccagaagttaagtttaactggtatgtggacggggtcgaggtgcacaatgctaaaacaaagcccagggaggagcaatataactccacatacagagtggtgtccgttctgacagtcctgcaccaggactggctgaacgggaaggaatacaagtgcaaggtgtctaataaggcactgccagcccccatagagaagacaatctctaaagctaaaggccaaccacgcgagcctcaggtctacacactgccaccatccagggacgaactgaccaagaatcaggtgagcctgacttgtctcgtcaaaggattctacccaagcgacatcgccgtggagtgggaatccaacggccaaccagagaacaactacaagaccaccccaccagtcctggactctgatgggagctttttcctgtattccaagctgacagtggacaagtctcggtggcaacagggcaacgtgttcagctgctccgtgatgcatgaagccctgcataaccactatacccagaaaagcctcagcctgtcccccgggaaataatgaattc

SEQ ID NO: 137 - DNA, 652 bp, Artificial Sequence
  m2B8 light chain(nucleotide)
gacattgtgatgacccagtctccatcttatcttgctgcatctcctggagaaaccattactataaattgcagggcaagtaagagcattagcaaatatttagcctggtatcgagagaaacctgggaaaactaataatcttcttatctactctggatccactttgcaatctggaattccatcaaggttcagtggcagtggatctggtacagatttcactctcaccatcagtagcctggagcctgaagattttgcaatgtattactgtcaacagcataatgaatacccgctcacgttcggtgctgggaccaagctggagctgaaacgtacggtggctgcaccatctgtcttcatcttcccgccatctgatgagcagttgaaatctggtaccgctagcgttgtgtgcctgctgaataacttttatccacgggaggctaaggtgcagtggaaagtggacaatgccctccagagcggaaatagccaagagtccgttaccgaacaggactctaaagactctacatactccctgtcctccacactgaccctctccaaggccgactatgagaaacacaaggtttacgcatgcgaggtcacacaccagggactctcctctcccgtgaccaagagcttcaaccggggagaatgctaatgaattc

SEQ ID NO: 138 - DNA, 1360 bp, Artificial Sequence
  m2B8 heavy chain(nucleotide)
gaggtgcagctgcaggagtctggtggaggattggtgcagcctaaagggtcattgaaactctcatgtgcagcctctggattcaacttcaatacctacaccatgaactgggtccgccaggctccaggaaagggtttggaatgggttgctcgcataagatataaaagtaataattatgcaacatattatgccgattcagtgaaagacagattcaccatctccagagatgattcagaaagcatcctctatctgcaaatgaacaacttgagaactgacgacacagccatttatttctgtgtgagggaactgggactgtggtacttcgatgtctggggcgcagggaccacggtcaccgtctcctcagccagcactaaggggccctctgtgtttccactcgccccttctagcaaaagcacttccggaggcactgcagcactcgggtgtctggtcaaagattatttccctgagccagtcaccgtgagctggaactctggcgccctcacctccggggttcacacctttccagccgtcctgcagtcctccggcctgtactccctgagcagcgtcgttaccgtgccatcctcttctctggggacccagacatacatctgcaatgtcaaccataagcctagcaacaccaaggtggacaaaaaggtcgagccaaagagctgcgataagacacacacctgccctccatgccccgcacctgaactcctgggcgggccttccgttttcctgtttcctcccaagcccaaggatacactgatgattagccgcacccccgaagtcacttgcgtggtggtggatgtgagccatgaagatccagaagttaagtttaactggtatgtggacggggtcgaggtgcacaatgctaaaacaaagcccagggaggagcaatataactccacatacagagtggtgtccgttctgacagtcctgcaccaggactggctgaacgggaaggaatacaagtgcaaggtgtctaataaggcactgccagcccccatagagaagacaatctctaaagctaaaggccaaccacgcgagcctcaggtctacacactgccaccatccagggacgaactgaccaagaatcaggtgagcctgacttgtctcgtcaaaggattctacccaagcgacatcgccgtggagtgggaatccaacggccaaccagagaacaactacaagaccaccccaccagtcctggactctgatgggagctttttcctgtattccaagctgacagtggacaagtctcggtggcaacagggcaacgtgttcagctgctccgtgatgcatgaagccctgcataaccactatacccagaaaagcctcagcctgtcccccgggaaataatgaattc

SEQ ID NO: 139 - DNA, 652 bp, Artificial Sequence
  m4H3 light chain(nucleotide)
gatatcgttctcacccagtctccagccatcctctctgtgagtccaggagaaagagtcagtttctcctgcagggccagtcagagcattggcacaagcatgcactggtatcagcaaagaaaaaatggttctccaaggcttctcataaagtatgcttctgagtctatctctgggatcccttccaggtttagtggcagtggatcagggacagattttactcttagcatcaacagtgtggagtctgaggatattgcagattattactgtcaacaaactaataactggccgtggacgttcggtggaggcaccaagctggaattcaaacgtacggtggctgcaccatctgtcttcatcttcccgccatctgatgagcagttgaaatctggtaccgctagcgttgtgtgcctgctgaataacttttatccacgggaggctaaggtgcagtggaaagtggacaatgccctccagagcggaaatagccaagagtccgttaccgaacaggactctaaagactctacatactccctgtcctccacactgaccctctccaaggccgactatgagaaacacaaggtttacgcatgcgaggtcacacaccagggactctcctctcccgtgaccaagagcttcaaccggggagaatgctaatgaattc

SEQ ID NO: 140 - DNA, 1363 bp, Artificial Sequence
  m4H3 heavy chain(nucleotide)
caggtgcagctgcagcagtctggacctgagctggtgaagcctggcgcttcagtgaagatatcctgcaaggcttctggttactcattcactgcctacaacattaactgggtgaagcagaccaatggaaagagccttgagtggattggaataattaatcctaactatggtactactagttacaaccagaagttcaagggcaaggccacattgactgtagaccaatcttccagtacagcctacatgcagctcaacagcctgacatctgaggactctgcagtctattactgtgcaagacggaatggtgactacgtgggatatgctatggactcctggggtcaaggaacctcagtcaccgtctcctcagccagcactaaggggccctctgtgtttccactcgccccttctagcaaaagcacttccggaggcactgcagcactcgggtgtctggtcaaagattatttccctgagccagtcaccgtgagctggaactctggcgccctcacctccggggttcacacctttccagccgtcctgcagtcctccggcctgtactccctgagcagcgtcgttaccgtgccatcctcttctctggggacccagacatacatctgcaatgtcaaccataagcctagcaacaccaaggtggacaaaaaggtcgagccaaagagctgcgataagacacacacctgccctccatgccccgcacctgaactcctgggcgggccttccgttttcctgtttcctcccaagcccaaggatacactgatgattagccgcacccccgaagtcacttgcgtggtggtggatgtgagccatgaagatccagaagttaagtttaactggtatgtggacggggtcgaggtgcacaatgctaaaacaaagcccagggaggagcaatataactccacatacagagtggtgtccgttctgacagtcctgcaccaggactggctgaacgggaaggaatacaagtgcaaggtgtctaataaggcactgccagcccccatagagaagacaatctctaaagctaaaggccaaccacgcgagcctcaggtctacacactgccaccatccagggacgaactgaccaagaatcaggtgagcctgacttgtctcgtcaaaggattctacccaagcgacatcgccgtggagtgggaatccaacggccaaccagagaacaactacaagaccaccccaccagtcctggactctgatgggagctttttcctgtattccaagctgacagtggacaagtctcggtggcaacagggcaacgtgttcagctgctccgtgatgcatgaagccctgcataaccactatacccagaaaagcctcagcctgtcccccgggaaataatgaattc

SEQ ID NO: 141 - DNA, 652 bp, Artificial Sequence
  m3E7 light chain(nucleotide)
gacattgtgatgacccaaactacagcaatcatgtctgcatttccaggggagaaggtcaccatgacctgcagtgccagctcaagtgtaagttacatgcactggtaccagcagaagtcaggcacctcccccaaaagatggatttatgacacatccaaactggcttctggagtccctgttcgcttcagtggcagtgggtctgggacctcttactctctcacaatcagcaacatggaggctgaagatgctgccacttattattgccagcagtggagtcgtaacccacccttcacgttcggtgctgggaccaagctggagctgaaacgtacggtggctgcaccatctgtcttcatcttcccgccatctgatgagcagttgaaatctggtaccgctagcgttgtgtgcctgctgaataacttttatccacgggaggctaaggtgcagtggaaagtggacaatgccctccagagcggaaatagccaagagtccgttaccgaacaggactctaaagactctacatactccctgtcctccacactgaccctctccaaggccgactatgagaaacacaaggtttacgcatgcgaggtcacacaccagggactctcctctcccgtgaccaagagcttcaaccggggagaatgctaatgaattc

SEQ ID NO: 142 - DNA, 1348 bp, Artificial Sequence
  m3E7 heavy chain(nucleotide)
cagatccagctggtgcagagcggaccagaactgaagaagccaggagagacagtcaagatctcctgcaaggcttctggatatacgttcacaacctatggaatgagctgggtgaaacaggctccaggaaagggtttgcactggatgggctggataaacacccactctggagcgccaacatatgttgatgacttcaagggacggtttgccttctctttggaaacctctgccagcactgcctttttgcagatcaacaacctcataaatgaggacacggctacatatttctgtgcaagagagggggatgctctggactactggggtcaaggaacctcagtcaccgtctcctcagccagcactaaggggccctctgtgtttccactcgccccttctagcaaaagcacttccggaggcactgcagcactcgggtgtctggtcaaagattatttccctgagccagtcaccgtgagctggaactctggcgccctcacctccggggttcacacctttccagccgtcctgcagtcctccggcctgtactccctgagcagcgtcgttaccgtgccatcctcttctctggggacccagacatacatctgcaatgtcaaccataagcctagcaacaccaaggtggacaaaaaggtcgagccaaagagctgcgataagacacacacctgccctccatgccccgcacctgaactcctgggcgggccttccgttttcctgtttcctcccaagcccaaggatacactgatgattagccgcacccccgaagtcacttgcgtggtggtggatgtgagccatgaagatccagaagttaagtttaactggtatgtggacggggtcgaggtgcacaatgctaaaacaaagcccagggaggagcaatataactccacatacagagtggtgtccgttctgacagtcctgcaccaggactggctgaacgggaaggaatacaagtgcaaggtgtctaataaggcactgccagcccccatagagaagacaatctctaaagctaaaggccaaccacgcgagcctcaggtctacacactgccaccatccagggacgaactgaccaagaatcaggtgagcctgacttgtctcgtcaaaggattctacccaagcgacatcgccgtggagtgggaatccaacggccaaccagagaacaactacaagaccaccccaccagtcctggactctgatgggagctttttcctgtattccaagctgacagtggacaagtctcggtggcaacagggcaacgtgttcagctgctccgtgatgcatgaagccctgcataaccactatacccagaaaagcctcagcctgtcccccgggaaataatgaattc

SEQ ID NO: 143 - DNA, 652 bp, Artificial Sequence
  m1A8 light chain(nucleotide)
gatattgtgctgacccagtctccagccatcctgtctgtgagtccaggagaaagagtcagtttctcctgcagggccagtcagagcattggcacaagcatacattggtatcagcaaagaacaaatggttctccaaggcttctcataaagtatgcttctgagtctatctctgggatcccttccaggtttagtggcagtggatcagggacagattttactcttagcatcaacagtgtggagtctgaagatattgcagattattactgtcaacaaagtaatagctggccactcacgttcggtgctgggaccaagctggagctgaaacgtacggtggctgcaccatctgtcttcatcttcccgccatctgatgagcagttgaaatctggtaccgctagcgttgtgtgcctgctgaataacttttatccacgggaggctaaggtgcagtggaaagtggacaatgccctccagagcggaaatagccaagagtccgttaccgaacaggactctaaagactctacatactccctgtcctccacactgaccctctccaaggccgactatgagaaacacaaggtttacgcatgcgaggtcacacaccagggactctcctctcccgtgaccaagagcttcaaccggggagaatgctaatgaattc

SEQ ID NO: 144 - DNA, 1366 bp, Artificial Sequence
  m1A8 heavy chain(nucleotide)
gaggtgcagctgcaggagtctggggctgaattggtaaagcctggggcttcagtgaagttgtcctgcaaggcttctggctacagtttcaccagctcctggatgcactgggtgaagcagaggcctggacaaggccttgagtggattggaatgattcatcctgatagtggttttactaactacaatgagaagttcaagagcaaggccacactgactgtagacaaatcctccagcacagcctacatgcgcctcagcagcctgacatctgaggactctgcggtctattactgtgcaaggacctcttactacgatactagctacacttctatggacttctggggtcaaggaaactcagtcaccgtctcctcagccagcactaaggggccctctgtgtttccactcgccccttctagcaaaagcacttccggaggcactgcagcactcgggtgtctggtcaaagattatttccctgagccagtcaccgtgagctggaactctggcgccctcacctccggggttcacacctttccagccgtcctgcagtcctccggcctgtactccctgagcagcgtcgttaccgtgccatcctcttctctggggacccagacatacatctgcaatgtcaaccataagcctagcaacaccaaggtggacaaaaaggtcgagccaaagagctgcgataagacacacacctgccctccatgccccgcacctgaactcctgggcgggccttccgttttcctgtttcctcccaagcccaaggatacactgatgattagccgcacccccgaagtcacttgcgtggtggtggatgtgagccatgaagatccagaagttaagtttaactggtatgtggacggggtcgaggtgcacaatgctaaaacaaagcccagggaggagcaatataactccacatacagagtggtgtccgttctgacagtcctgcaccaggactggctgaacgggaaggaatacaagtgcaaggtgtctaataaggcactgccagcccccatagagaagacaatctctaaagctaaaggccaaccacgcgagcctcaggtctacacactgccaccatccagggacgaactgaccaagaatcaggtgagcctgacttgtctcgtcaaaggattctacccaagcgacatcgccgtggagtgggaatccaacggccaaccagagaacaactacaagaccaccccaccagtcctggactctgatgggagctttttcctgtattccaagctgacagtggacaagtctcggtggcaacagggcaacgtgttcagctgctccgtgatgcatgaagccctgcataaccactatacccagaaaagcctcagcctgtcccccgggaaataatgaattc

SEQ ID NO: 145 - DNA, 321 bp, Artificial Sequence; identical to SEQ ID NO: 54
  m4G1 light chain(nucleotide)

SEQ ID NO: 146 - DNA, 1369 bp, Artificial Sequence
  m4G1 heavy chain(nucleotide)
caggtccagctgcagcagtccggacctgagctggtgaagcctggcgcttcagtgaagatatcatgcaaggcttctggttactcattcactgcctacaacatgaactgggtgaagcagagcaagggaaagagccttgagtggattggactaattaatcctaactatgccacgactagttacaatcagaagttcaaggacaaggccacattgactgtggaccaatcttccagcacagcctacatgcagctcaacagcctgacatctgaggactctgcagtctattactgtgcctactatagttactatagttacggggggggatatgctatggactactggggtcaaggaacctcagtcaccgtctcctcagccagcactaaggggccctctgtgtttccactcgccccttctagcaaaagcacttccggaggcactgcagcactcgggtgtctggtcaaagattatttccctgagccagtcaccgtgagctggaactctggcgccctcacctccggggttcacacctttccagccgtcctgcagtcctccggcctgtactccctgagcagcgtcgttaccgtgccatcctcttctctggggacccagacatacatctgcaatgtcaaccataagcctagcaacaccaaggtggacaaaaaggtcgagccaaagagctgcgataagacacacacctgccctccatgccccgcacctgaactcctgggcgggccttccgttttcctgtttcctcccaagcccaaggatacactgatgattagccgcacccccgaagtcacttgcgtggtggtggatgtgagccatgaagatccagaagttaagtttaactggtatgtggacggggtcgaggtgcacaatgctaaaacaaagcccagggaggagcaatataactccacatacagagtggtgtccgttctgacagtcctgcaccaggactggctgaacgggaaggaatacaagtgcaaggtgtctaataaggcactgccagcccccatagagaagacaatctctaaagctaaaggccaaccacgcgagcctcaggtctacacactgccaccatccagggacgaactgaccaagaatcaggtgagcctgacttgtctcgtcaaaggattctacccaagcgacatcgccgtggagtgggaatccaacggccaaccagagaacaactacaagaccaccccaccagtcctggactctgatgggagctttttcctgtattccaagctgacagtggacaagtctcggtggcaacagggcaacgtgttcagctgctccgtgatgcatgaagccctgcataaccactatacccagaaaagcctcagcctgtcccccgggaaataatgaattc

SEQ ID NO: 147 - DNA, 649 bp, Artificial Sequence
  m2G3 light chain(nucleotide)
gatatcgtgctcactcagtctccagcaatcatgtctgcatctccaggggagaaggtcaccatgacctgcagtgccagctcaagtgtaagttacatgaactggtaccagcagaagtcaggcacctcccccaaaagatggatttatgacacatccaaactggcttctggagtccctgttcgcttcagtggcagtgggtctgggacctcttactctctcacaatcagcagcatggaggctgaagatgctgccacttattactgccagcagtggaatagtaacccacccacgttcggtgctgggaccaagctggagctgaaacgtacggtggctgcaccatctgtcttcatcttcccgccatctgatgagcagttgaaatctggtaccgctagcgttgtgtgcctgctgaataacttttatccacgggaggctaaggtgcagtggaaagtggacaatgccctccagagcggaaatagccaagagtccgttaccgaacaggactctaaagactctacatactccctgtcctccacactgaccctctccaaggccgactatgagaaacacaaggtttacgcatgcgaggtcacacaccagggactctcctctcccgtgaccaagagcttcaaccggggagaatgctaatgaattc

SEQ ID NO: 148 - DNA, 1351 bp, Artificial Sequence
  m2G3 heavy chain(nucleotide)
gaggtgaagctgcaggagtctgggggaggcttagtgaagcctggagggtccctgaaactctcctgtgcagcctctggattcactttcagtagctttgccatgtcttggattcgccagactccggaaaagaggctggagtgggtcgcggccattagtgatggtggtacttacacctactatccaaacaatgtaaagggccgattcaccatctccagagacgatgccaagaataacctgtacctgcaaatgagtcatctgaagtctgaggacacagccatgtattactgtgtaagaaatagggggggaccctttgactactggggccaaggcaccactctcacagtctcctcagccagcactaaggggccctctgtgtttccactcgccccttctagcaaaagcacttccggaggcactgcagcactcgggtgtctggtcaaagattatttccctgagccagtcaccgtgagctggaactctggcgccctcacctccggggttcacacctttccagccgtcctgcagtcctccggcctgtactccctgagcagcgtcgttaccgtgccatcctcttctctggggacccagacatacatctgcaatgtcaaccataagcctagcaacaccaaggtggacaaaaaggtcgagccaaagagctgcgataagacacacacctgccctccatgccccgcacctgaactcctgggcgggccttccgttttcctgtttcctcccaagcccaaggatacactgatgattagccgcacccccgaagtcacttgcgtggtggtggatgtgagccatgaagatccagaagttaagtttaactggtatgtggacggggtcgaggtgcacaatgctaaaacaaagcccagggaggagcaatataactccacatacagagtggtgtccgttctgacagtcctgcaccaggactggctgaacgggaaggaatacaagtgcaaggtgtctaataaggcactgccagcccccatagagaagacaatctctaaagctaaaggccaaccacgcgagcctcaggtctacacactgccaccatccagggacgaactgaccaagaatcaggtgagcctgacttgtctcgtcaaaggattctacccaagcgacatcgccgtggagtgggaatccaacggccaaccagagaacaactacaagaccaccccaccagtcctggactctgatgggagctttttcctgtattccaagctgacagtggacaagtctcggtggcaacagggcaacgtgttcagctgctccgtgatgcatgaagccctgcataaccactatacccagaaaagcctcagcctgtcccccgggaaataatgaattc

SEQ ID NO: 149 - DNA, 649 bp, Artificial Sequence
  m2F11 light chain(nucleotide)
gatatcgtgctcacccaaactccagcactcatgtctgcatctccaggggagaaggtcaccatgacctgcagtgccagctcaagtgtaggttccatgcactggtaccagcagaagtcaggcacctcccccaaaagatggatttatgacacatccaaactggcttctggagtccctgctcgcttcagtggcagtgggtctgggacctcttactctctcacaatcagcagcatggaggctgaagatgctgccacttattactgccaacagtggagtagtatcccacccacgttcggtgctgggaccacgctggagctgaaacgtacggtggctgcaccatctgtcttcatcttcccgccatctgatgagcagttgaaatctggtaccgctagcgttgtgtgcctgctgaataacttttatccacgggaggctaaggtgcagtggaaagtggacaatgccctccagagcggaaatagccaagagtccgttaccgaacaggactctaaagactctacatactccctgtcctccacactgaccctctccaaggccgactatgagaaacacaaggtttacgcatgcgaggtcacacaccagggactctcctctcccgtgaccaagagcttcaaccggggagaatgctaatgaattc

SEQ ID NO: 150 - DNA, 1351 bp, Artificial Sequence
  m2F11 heavy chain(nucleotide)
gaggtgcagctgcaggagtctgggggagacttagtgaagcctggagggtccctgaaactctcctgtgcagcctctggattcactttcagtagctatgccatgtcttgggttcgccagactccggaaaagaggctggagtgggtcgcaatcattggtgatggtgatacttacacctactatccagacagtgtaaagggccgattcaccgtctccagagacaatgccaagaacaacctctacctgcaaatgagccatctgaagtctgaggacacagccatgtattactgtgtaagaactagggggggaccctttgactactggggccaaggcaccactctcacagtctcctcagccagcactaaggggccctctgtgtttccactcgccccttctagcaaaagcacttccggaggcactgcagcactcgggtgtctggtcaaagattatttccctgagccagtcaccgtgagctggaactctggcgccctcacctccggggttcacacctttccagccgtcctgcagtcctccggcctgtactccctgagcagcgtcgttaccgtgccatcctcttctctggggacccagacatacatctgcaatgtcaaccataagcctagcaacaccaaggtggacaaaaaggtcgagccaaagagctgcgataagacacacacctgccctccatgccccgcacctgaactcctgggcgggccttccgttttcctgtttcctcccaagcccaaggatacactgatgattagccgcacccccgaagtcacttgcgtggtggtggatgtgagccatgaagatccagaagttaagtttaactggtatgtggacggggtcgaggtgcacaatgctaaaacaaagcccagggaggagcaatataactccacatacagagtggtgtccgttctgacagtcctgcaccaggactggctgaacgggaaggaatacaagtgcaaggtgtctaataaggcactgccagcccccatagagaagacaatctctaaagctaaaggccaaccacgcgagcctcaggtctacacactgccaccatccagggacgaactgaccaagaatcaggtgagcctgacttgtctcgtcaaaggattctacccaagcgacatcgccgtggagtgggaatccaacggccaaccagagaacaactacaagaccaccccaccagtcctggactctgatgggagctttttcctgtattccaagctgacagtggacaagtctcggtggcaacagggcaacgtgttcagctgctccgtgatgcatgaagccctgcataaccactatacccagaaaagcctcagcctgtcccccgggaaataatgaattc

SEQ ID NO: 151 - DNA, 664 bp, Artificial Sequence
  m3B8 light chain(nucleotide)
gatatcgtgctgacccaatctccagcttctttggctgtgtctctagggcagagagccaccatctcctgcagagccagtgaaagtgttgaatattatggcacaagtttaatgcagtggtaccaacagaaaccaggacagccacccaaactcctcatctatgctgcatccaacgtagaatctggggtccctgccaggtttagtggcagtgggtctgggacagacttcagcctcaacatccatcctgtggaggaggatgattttgcaatgtatttctgtcagcaaagtaggaagattccttacacgttcggaggggggaccaagctggaaataaaacgtacggtggctgcaccatctgtcttcatcttcccgccatctgatgagcagttgaaatctggtaccgctagcgttgtgtgcctgctgaataacttttatccacgggaggctaaggtgcagtggaaagtggacaatgccctccagagcggaaatagccaagagtccgttaccgaacaggactctaaagactctacatactccctgtcctccacactgaccctctccaaggccgactatgagaaacacaaggtttacgcatgcgaggtcacacaccagggactctcctctcccgtgaccaagagcttcaaccggggagaatgctaatgaattc

SEQ ID NO: 152 - DNA, 1363 bp, Artificial Sequence
  m3B8 heavy chain(nucleotide)
caggtccagctgcaggagtcaggacctggcctggtggcgccctcacagagcctgtccatcacatgcactgtctcagggttctcattaaccaactatgctgtaagctgggttcgccagcctccaggaaagggtctggagtggctgggagtaatatggggtgacgggaccacaaattatcattcagctctcatatccagactgattatcagcaaggataactccaagagccaagttttcttaaaactgaacagtctgcaaactgatgacacagccacgtactactgtgccaaagagggcgactatggtgactacgtaggctggtttgcttactggggccaagggactctggtcactgtctctgcagccagcactaaggggccctctgtgtttccactcgccccttctagcaaaagcacttccggaggcactgcagcactcgggtgtctggtcaaagattatttccctgagccagtcaccgtgagctggaactctggcgccctcacctccggggttcacacctttccagccgtcctgcagtcctccggcctgtactccctgagcagcgtcgttaccgtgccatcctcttctctggggacccagacatacatctgcaatgtcaaccataagcctagcaacaccaaggtggacaaaaaggtcgagccaaagagctgcgataagacacacacctgccctccatgccccgcacctgaactcctgggcgggccttccgttttcctgtttcctcccaagcccaaggatacactgatgattagccgcacccccgaagtcacttgcgtggtggtggatgtgagccatgaagatccagaagttaagtttaactggtatgtggacggggtcgaggtgcacaatgctaaaacaaagcccagggaggagcaatataactccacatacagagtggtgtccgttctgacagtcctgcaccaggactggctgaacgggaaggaatacaagtgcaaggtgtctaataaggcactgccagcccccatagagaagacaatctctaaagctaaaggccaaccacgcgagcctcaggtctacacactgccaccatccagggacgaactgaccaagaatcaggtgagcctgacttgtctcgtcaaaggattctacccaagcgacatcgccgtggagtgggaatccaacggccaaccagagaacaactacaagaccaccccaccagtcctggactctgatgggagctttttcctgtattccaagctgacagtggacaagtctcggtggcaacagggcaacgtgttcagctgctccgtgatgcatgaagccctgcataaccactatacccagaaaagcctcagcctgtcccccgggaaataatgaattc